European Patent Specification EP 3 583 953 B1, published June 28, 2023. Title: Optimierte Injektionsformulierung für mRNA. Applicant: CureVac AG. Application PCT/EP2006/004784. The sequence listing filed with the application follows.

SEQUENCE LISTING (34 sequences)

SEQ ID NO: 1 - RNA, 13 nt, Unknown
  Kozak-Sequenz (siehe Beschreibung Seite 16)
gccgccaccaugg

SEQ ID NO: 2 - RNA, 15 nt, Unknown
  Stabilisierungssequenz der allgemeinen Formel (C/U)CCANxCCC(U/A)PyxUC(C/U)CC (siehe Beschreibung Seite 18)
  misc_feature (1)..(1): n = c oder u
  misc_feature (5)..(5): n = a, c, u, g oder andere
  repeat_unit (5)..(5): x = beliebig
  misc_feature (9)..(9): n = u oder a
  repeat_unit (10)..(10): x = beliebig
  misc_feature (10)..(10): n = Py (Pyrimidin)
  misc_feature (13)..(13): n = c oder u
nccancccnnucncc

SEQ ID NO: 3 - RNA, 75 nt, Artificial
  Beschreibung der Sequenz: Signalsequenz HLA-B*07022
  CDS (1)..(75)
augcuggugauggccccgcggaccguccuccugcugcugagcgcggcccuggcccugacggagaccugggccggc

SEQ ID NO: 4 - protein, 25 aa, Artificial
  Synthetic Construct
MLVMAPRTVLLLLSAALALTETWAG

SEQ ID NO: 5 - RNA, 75 nt, Artificial
  Beschreibung der Sequenz: Signalsequenz HLA-A*3202
  CDS (1)..(75)
auggccgugauggcgccgcggacccugcuccugcugcugcugggcgcccuggcccucacgcagaccugggccggg

SEQ ID NO: 6 - protein, 25 aa, Artificial
  Synthetic Construct
MAVMAPRTLLLLLLGALALTQTWAG

SEQ ID NO: 7 - RNA, 75 nt, Artificial
  Beschreibung der Sequenz: Signalsequenz HLA-A*01011
  CDS (1)..(75)
auggccgugauggcgccgcggacccugcuccugcugcugagcggcgcccuggcccugacgcagaccugggccggg

SEQ ID NO: 8 - protein, 25 aa, Artificial
  Synthetic Construct
MAVMAPRTLLLLLSGALALTQTWAG

SEQ ID NO: 9 - RNA, 75 nt, Artificial; identical to SEQ ID NO: 7
  Beschreibung der Sequenz: Signalsequenz HLA-A*0102
  CDS (1)..(75)

SEQ ID NO: 10 - protein, 25 aa, Artificial
  Synthetic Construct
MAVMAPRTLLLLLSGALALTQTWAG

SEQ ID NO: 11 - RNA, 75 nt, Artificial
  Beschreibung der Sequenz: Signalsequenz HLA-A*0201
  CDS (1)..(75)
auggccgugauggcgccgcggacccugguccuccugcugagcggcgcccuggcccugacgcagaccugggccggg

SEQ ID NO: 12 - protein, 25 aa, Artificial
  Synthetic Construct
MAVMAPRTLVLLLSGALALTQTWAG

SEQ ID NO: 13 - RNA, 75 nt, Artificial; identical to SEQ ID NO: 7
  Beschreibung der Sequenz: Signalsequenz HLA-A*0301
  CDS (1)..(75)

SEQ ID NO: 14 - protein, 25 aa, Artificial
  Synthetic Construct
MAVMAPRTLLLLLSGALALTQTWAG

SEQ ID NO: 15 - RNA, 75 nt, Artificial; identical to SEQ ID NO: 7
  Beschreibung der Sequenz: Signalsequenz HLA-A*1101
  CDS (1)..(75)

SEQ ID NO: 16 - protein, 25 aa, Artificial
  Synthetic Construct
MAVMAPRTLLLLLSGALALTQTWAG

SEQ ID NO: 17 - RNA, 75 nt, Artificial; identical to SEQ ID NO: 3
  Beschreibung der Sequenz: Signalsequenz HLA-B*070201
  CDS (1)..(75)

SEQ ID NO: 18 - protein, 25 aa, Artificial
  Synthetic Construct
MLVMAPRTVLLLLSAALALTETWAG

SEQ ID NO: 19 - RNA, 75 nt, Artificial
  Beschreibung der Sequenz: Signalsequenz HLA-B*2702
  CDS (1)..(75)
augcgggugaccgccccgcgcacgcugcuccugcugcuguggggcgcggucgcccugaccgagaccugggccggg

SEQ ID NO: 20 - protein, 25 aa, Artificial
  Synthetic Construct
MRVTAPRTLLLLLWGAVALTETWAG

SEQ ID NO: 21 - RNA, 78 nt, Artificial
  Beschreibung der Sequenz: Signalsequenz HLA-Cw*010201
  CDS (1)..(78)
augcgggugauggccccgcgcacccugauccuccugcugagcggcgcgcuggcccugacggagaccugggccugcucg

SEQ ID NO: 22 - protein, 26 aa, Artificial
  Synthetic Construct
MRVMAPRTLILLLSGALALTETWACS

SEQ ID NO: 23 - RNA, 78 nt, Artificial
  Beschreibung der Sequenz: Signalsequenz HLA-Cw*02021
  CDS (1)..(78)
augcgggugauggccccgcgcacccugcuccugcugcugagcggcgcgcuggcccugacggagaccugggccugcucg

SEQ ID NO: 24 - protein, 26 aa, Artificial
  Synthetic Construct
MRVMAPRTLLLLLSGALALTETWACS

SEQ ID NO: 25 - RNA, 75 nt, Artificial
  Beschreibung der Sequenz: Signalsequenz HLA-E*0101
  CDS (1)..(75)
augguggacggcacccugcuccugcugagcucggaggcccuggcgcugacgcagaccugggccgggagccacagc

SEQ ID NO: 26 - protein, 25 aa, Artificial
  Synthetic Construct
MVDGTLLLLSSEALALTQTWAGSHS

SEQ ID NO: 27 - RNA, 87 nt, Artificial
  Beschreibung der Sequenz: Signalsequenz HLA-DRB1
  CDS (1)..(87)
auggugugccugaagcucccgggcgggagcugcaugaccgcccugacggucacccugauggugcugucgagcccccuggcgcuggcc

SEQ ID NO: 28 - protein, 29 aa, Artificial
  Synthetic Construct
MVCLKLPGGSCMTALTVTLMVLSSPLALA

SEQ ID NO: 29 - RNA, 75 nt, Artificial
  Beschreibung der Sequenz: Signalsequenz HLA-DRA1
  CDS (1)..(75)
auggccaucagcggcgugccgguccugggguucuucaucaucgcggugcucaugucggcccaggagagcugggcc

SEQ ID NO: 30 - protein, 25 aa, Artificial
  Synthetic Construct
MAISGVPVLGFFIIAVLMSAQESWA

SEQ ID NO: 31 - RNA, 87 nt, Artificial
  Beschreibung der Sequenz: Signalsequenz HLA-DR4
  CDS (1)..(87)
auggugugccugaaguucccgggcgggagcugcauggccgcgcucaccgucacgcugauggugcugucgagcccccuggcccuggcc

SEQ ID NO: 32 - protein, 29 aa, Artificial
  Synthetic Construct
MVCLKFPGGSCMAALTVTLMVLSSPLALA

SEQ ID NO: 33 - RNA, 87 nt, Artificial
  Myelin oligodendroocyte glycoprotein (siehe Beschreibung Seite 21)
  CDS (1)..(87)
auggccugccuguggagcuucucguggccgagcugcuuccucagccugcugcugcugcugcuccugcagcugagcugcagcuacgcg

SEQ ID NO: 34 - protein, 29 aa, Artificial
  Synthetic Construct
MACLWSFSWPSCFLSLLLLLLLQLSCSYA